European Patent Application EP 4 520 827 A1, published March 12, 2025. Title: 一种环状RNA-circ-Magi1及其应用. Applicant: 源生生物科技（青岛）有限责任公司. The sequence listing filed with the application follows.

SEQUENCE LISTING (20 sequences)

SEQ ID NO: 1 - RNA, 327 nt, synthetic construct
  source 1..327: mol_type = other RNA
gcacaacccgatctcccagagaaggagaagtgcctggcgtggactataactttctgactgtgaaggagttcttggacctcgagcagagtgggactcttctggaagtcggcacctatgaaggaaactattatgggacacccaagcctcctagccagccagtcagtgggaaagtgatcacgacggatgccttgcacagccttcagtctggctctaagcagtcgaccccgaagcgaaccaagtcctacaatgatatgcaaaatgctggcatagtccacgcggagaatgaggaggaggatgacgttcctgaaatgaacagcagctttacag

SEQ ID NO: 2 - DNA, 20 bp, synthetic construct
  source 1..20: mol_type = other DNA
tctgctcgaggtccaagaac

SEQ ID NO: 3 - DNA, 22 bp, synthetic construct
  source 1..22: mol_type = other DNA
cagcagctttacaggcacaacc

SEQ ID NO: 4 - RNA, 327 nt, synthetic construct
  source 1..327: mol_type = other RNA
gcacaacccggtctcccagagaaggagaagtgcctggtgtggattacagctttctgactgtgaaggagttcttggacctcgagcagagcgggaccctgttggaagtcggcacctatgaaggaaactattatgggacacccaaacctcctagccagccagtcagtgggaaagtgatcacgacggatgccttgcacagcctgcagtctggctccaagcagtcgacccctaagcgaacaaagtcctacaatgatatgcaaaatgctggcatagtccacccggagaatgaggaggaggaggatgtccctgaaatgaacagtagctttacag

SEQ ID NO: 5 - DNA, 20 bp, synthetic construct
  source 1..20: mol_type = other DNA
tctgctcgaggtccaagaac

SEQ ID NO: 6 - DNA, 22 bp, synthetic construct
  source 1..22: mol_type = other DNA
cagtagctttacaggcacaacc

SEQ ID NO: 7 - RNA, 19 nt, synthetic construct
  source 1..19: mol_type = other RNA
gctttacaggcacaacccg

SEQ ID NO: 8 - RNA, 59 nt, synthetic construct
  source 1..59: mol_type = other RNA
aattcgctttacaggcacaacccgttcaagagacgggttgtgcctgtaaagcttttttg

SEQ ID NO: 9 - RNA, 59 nt, synthetic construct
  source 1..59: mol_type = other RNA
gatccaaaaaagctttacaggcacaacccgtctcttgaacgggttgtgcctgtaaagcg

SEQ ID NO: 10 - RNA, 21 nt, synthetic construct
  source 1..21: mol_type = other RNA
ttctccgaacgtgtcacgtaa

SEQ ID NO: 11 - RNA, 64 nt, synthetic construct
  source 1..64: mol_type = other RNA
gatccgttctccgaacgtgtcacgtaattcaagagattacgtgacacgttcggagaattttttc

SEQ ID NO: 12 - RNA, 64 nt, synthetic construct
  source 1..64: mol_type = other RNA
aattgaaaaaattctccgaacgtgtcacgtaatctcttgaattacgtgacacgttcggagaacg

SEQ ID NO: 13 - RNA, 21 nt, synthetic construct
  source 1..21: mol_type = other RNA
gctttacaggcacaacccgtt

SEQ ID NO: 14 - RNA, 21 nt, synthetic construct
  source 1..21: mol_type = other RNA
cgggttgtgcctgtaaagctt

SEQ ID NO: 15 - RNA, 21 nt, synthetic construct
  source 1..21: mol_type = other RNA
ttctccgaacgtgtcacgttt

SEQ ID NO: 16 - RNA, 21 nt, synthetic construct
  source 1..21: mol_type = other RNA
acgtgacacgttcggagaatt

SEQ ID NO: 17 - RNA, 27 nt, synthetic construct
  source 1..27: mol_type = other RNA
gactcttctggaagtcggcacctattt

SEQ ID NO: 18 - RNA, 27 nt, synthetic construct
  source 1..27: mol_type = other RNA
ataggtgccgacttccagaagagtctt

SEQ ID NO: 19 - RNA, 27 nt, synthetic construct
  source 1..27: mol_type = other RNA
actcttctggaagtcggcacctatgtt

SEQ ID NO: 20 - RNA, 27 nt, synthetic construct
  source 1..27: mol_type = other RNA
cataggtgccgacttccagaagagttt